European Patent Application EP 4 502 160 A1, published February 5, 2025. Title: Proteins with alpha 1,2-fucosyltransferase activity and method for the production of lacto- N-fucopentaose I (LNFPI). Applicant: キリンホールディングス株式会社. Application JP. The sequence listing filed with the application follows.

SEQUENCE LISTING (95 sequences)

SEQ ID NO: 1 - DNA, 903 bp, Gramella sp. MAR_2010_147
  source 1..903: mol_type = genomic DNA
atgagcaagaagaagccggttatcattgagatcctgggtggtatcggtaatcagatgtttcagtttgcgctggcgaaaatcctggcggagaagaacgacagcgaactgttcatcgacaccaacttctacaaggagaccagccaaaacctgaagaacttcccgcgttacttcagcgttggtatcttcgacctgcagttcaagctggcgaccgaaaaggagaaaatctttttcaaacacccgagcctgaaaaaccgtctgaaccgtaaactgggtctgaactatccgaaggtgttcaaagagaagagctttaacttcgatccggagctgctgaccatgaaagcgccgatcttcctgaagggctactttcagagctacaagtatttcgcgggtaccgaaagcaagatccgtcagctgtacgagttcccggatgagaagctggacagccgtaacgaagagatcaagaaccgtattatcaccaaaaccagcgttagcgttcacatccgtcgtggtgattacgtggagaaccgtaaaacccaggactttcacggtaactgcagcgtggagtactacaagaaagcggttgagtatctgagcgcgaccatcaaggacttcaacctggtgttctttagcgatgacattgcgtgggttcaaaaccagttcaaagacctgccgtacgagaagaaattcgttaccggtaacctgtacgagaacagctggaaagatatgtacctgatgagcctgtgcgatcacaacatcattgcgaacagcagcttcagctggtgggcggcgtggctgaacaagaacccggaaaagaaggtggttgcgccgaagaaatggtttgcggacatggaccaagaacaaaagagcctggacctgctgccgccggactgggtgcgtatctaa

SEQ ID NO: 2 - protein, 300 aa, Gramella sp. MAR_2010_147
MSKKKPVIIEILGGIGNQMFQFALAKILAEKNDSELFIDTNFYKETSQNLKNFPRYFSVGIFDLQFKLATEKEKIFFKHPSLKNRLNRKLGLNYPKVFKEKSFNFDPELLTMKAPIFLKGYFQSYKYFAGTESKIRQLYEFPDEKLDSRNEEIKNRIITKTSVSVHIRRGDYVENRKTQDFHGNCSVEYYKKAVEYLSATIKDFNLVFFSDDIAWVQNQFKDLPYEKKFVTGNLYENSWKDMYLMSLCDHNIIANSSFSWWAAWLNKNPEKKVVAPKKWFADMDQEQKSLDLLPPDWVRI

SEQ ID NO: 3 - DNA, 843 bp, Francisella sp. FSC1006
  source 1..843: mol_type = genomic DNA
atgaaagttgtgaaaatccaaggtggtctgggtaatcaaatgttccaatatgcgttctacatgagcctgaagcaaaagtataaagattgctgcatcgacattcgtgactttgagacctatacccagcacaacggtttcgaactggaccgtgtgttcgagaacatccgtcagagcattagcctgtgccgttgcaagcgtaaattctttcgtagcctgttcagcaagtttctgaaccgttttatcaagtaccacaagaactactttagccaggatgacttcggtttcaacaagaaatactataacaaggacaactgctacctggatggttactggcagagcgaaaagtacttcaagagcgtggagaagcaaatccgtgagatttttaagttccagaccctggatgacaaaaacgcgaagatcctggaagagtacaagaaccgtagcctggttagcatccacgtgcgtcgtggtgattacatcaaccacccgctgcacggcgatatctgcaacctggattattacaacaacgcgattgacatcatcaagagccgtgtggagagcccgcactttttcgtgttcagcgatgacatcgaatggtgcaagcaatgcctggacatcgaggatgtgacctacatttgcaccaacaccggtagcgatagctaccgtgatatgcagattatgagcatctgcaagcacaacatcattgcgaacagcagcttcagctggtggggcgcgtggctgaaccagaacagcgagaagatcatcattgcgccgaaccgttggttcaacgacgatagcatcaatcagagcgacatctgcccggaaagctggatcaaaatctaa

SEQ ID NO: 4 - protein, 280 aa, Francisella sp. FSC1006
MKVVKIQGGLGNQMFQYAFYMSLKQKYKDCCIDIRDFETYTQHNGFELDRVFENIRQSISLCRCKRKFFRSLFSKFLNRFIKYHKNYFSQDDFGFNKKYYNKDNCYLDGYWQSEKYFKSVEKQIREIFKFQTLDDKNAKILEEYKNRSLVSIHVRRGDYINHPLHGDICNLDYYNNAIDIIKSRVESPHFFVFSDDIEWCKQCLDIEDVTYICTNTGSDSYRDMQIMSICKHNIIANSSFSWWGAWLNQNSEKIIIAPNRWFNDDSINQSDICPESWIKI

SEQ ID NO: 5 - DNA, 840 bp, Neisseriaceae bacterium DSM 100970
  source 1..840: mol_type = genomic DNA
atgcaaatcgtgtggtgcctgggcggtctgggtaatcaaatgttccaatatgcgttctatcgtaaactggagctgatgggtaaagaggtttacctggacctgagcgagttcaacaactacgatctgcacaacggtttcgaactgcagaagatctttgcggttgcgccgaagattatcccgagcattgcggttaagaaattccgtcagaacaagttctttaaagttctggcgcgtctgaagctgtaccagcgtatcatcagccagagcgaattcaactttaacagcaagtacctggactacagcttcagccgttacctgatcggttactggcaaagcgaaagctacttcgcggagatcgaacgtcagatccgtgaagacttcacctttccgagcctggatgcggcgaaccaactgatcgcgaaccagattcgtagcaccaacgcgattagcctgcacgttcgtatgggtgactacgtgaaccacccgctgcacggcggtatctgcaccaaagagttctacctgcgtgcgattgacatcattaaggacaaagtggagggtccgcagtttttcgtgttcagcaacgaaatcgactggtgcaagaacaacctgccgctggcgaacgcggtgtacgttggtggcaacgacggtgaaaacagctaccgtgacatgcagctgatgagcctgtgcaaacacaacatcattgcgaacagcagcttcagctggtggggtgcgtggctgaacagcaacatcaacaagattgtgatcgcgccggcgaagtggtttaacgatccgcaaatcaataccagcgacctgctgccggcgagctgggtgaaaatctaa

SEQ ID NO: 6 - protein, 279 aa, Neisseriaceae bacterium DSM 100970
MQIVWCLGGLGNQMFQYAFYRKLELMGKEVYLDLSEFNNYDLHNGFELQKIFAVAPKIIPSIAVKKFRQNKFFKVLARLKLYQRIISQSEFNFNSKYLDYSFSRYLIGYWQSESYFAEIERQIREDFTFPSLDAANQLIANQIRSTNAISLHVRMGDYVNHPLHGGICTKEFYLRAIDIIKDKVEGPQFFVFSNEIDWCKNNLPLANAVYVGGNDGENSYRDMQLMSLCKHNIIANSSFSWWGAWLNSNINKIVIAPAKWFNDPQINTSDLLPASWVKI

SEQ ID NO: 7 - DNA, 879 bp, Methylobacter tundripaludum
  source 1..879: mol_type = genomic DNA
atggttattacccatctgatcggcggtctgggcaatcaaatgtttcagtatgcggcgggtcgtgcggttagcctggagcgtggcgtgagcctgagcctggacattagcggtttcgcgaactacggtctgcaccagggtttcgaactgcagcgtatcttcaactgcaccgcggagattgcgaacgaggcggatgttcgtggtattctgggttggcaaagcagcccgcgtatccgtcaactgctgagccgtcaaaacatggcgatcttccgtcgtgagggttttgtggttgaaccgcacttccactactggcagggtatcaagagcgttccgcgtgactgctatctgaccggttactggcaaagcgaacagtacttcctggaagcggcggcgcaaattcgtgcggatttcacctttaaactgccgctggacaaccagaacatcgaactggcgaagcagattaacgcggtgaacgcggttagcctgcacgttcgtcgtggtgactatgcgaacaccccggaaaccaccgcgacccacggtctgtgcagcctggactattaccgtgttgcgattcgtcacatcgcggaacaagtgcagcaaccgcactttttcgtgtttagcgatgacattgcgtgggtgaagaacaacctgagcatcgactttccgtgccagtacgttgaccacaaccaaggcgcggagagctacaacgacatgcgtctgatgagcatgtgccgtcaccacatcattgcgaacagcagctttagctggtggggtgcgtggctgaacccgaacgttaacaagattgtggttgcgccgagccgttggttcgcgaaacagaccgatgtgcgtgacctgctgccgcaaggctggattaaacaataa

SEQ ID NO: 8 - protein, 292 aa, Methylobacter tundripaludum
MVITHLIGGLGNQMFQYAAGRAVSLERGVSLSLDISGFANYGLHQGFELQRIFNCTAEIANEADVRGILGWQSSPRIRQLLSRQNMAIFRREGFVVEPHFHYWQGIKSVPRDCYLTGYWQSEQYFLEAAAQIRADFTFKLPLDNQNIELAKQINAVNAVSLHVRRGDYANTPETTATHGLCSLDYYRVAIRHIAEQVQQPHFFVFSDDIAWVKNNLSIDFPCQYVDHNQGAESYNDMRLMSMCRHHIIANSSFSWWGAWLNPNVNKIVVAPSRWFAKQTDVRDLLPQGWIKQ

SEQ ID NO: 9 - DNA, 864 bp, Amphritea japonica
  source 1..864: mol_type = genomic DNA
atggtgaaaatcaaaatcatcggtggtctgggcaatcaaatgttccaatatgcggcggcgaagagcctggcggttctgaataatacccgtgttagcgcgaacgtgagcgttttcagcaactacaaaacccacccgctgcgtctgaacaaactgaactgcgactgcgaatttgacttcacccgtgacttccgtctggtgctgagcggctttccgctgctgggcagcgcgttcagcaagaaaagcatgctgctgaaccactacgtggaaaaggacctgctgtttgacagcagctttttcgacctggatgacaacgtgctgctgagcggttacttccagagcgagaagtacttcagcaacatccgtgagctgctgattcaggaattcagcctggacgatcgtctgaccgaagcggagctggcgatcaacaacaagatcgagagctgcaacagcatcgcgattcacatccgtcgtggtgattacatcaccgacctgagcgcgaacaacatccacggcatttgcagcgaggaatacttcgagaaagcgctgaactacctggacagcatcaacgtgctgagcgatccgaccaccaccctgttcatctttagcgacgatatcctgtggtgcaaggacaacctggcgttcaaatatcgtaccgtgttcgttgagggtagcgttgaccgtccggaagtggatatccacctgatgagcaaatgcaagcaccaagtgatcagcaacagcacctttagctggtggggtgcgtggctgaacaccaacctggacaagtgcgttatcgcgccgctgaaatggtttaatagcctgcacgatagcaccgacattgttccgaagcagtggatgcgtctgtaa

SEQ ID NO: 10 - protein, 287 aa, Amphritea japonica
MVKIKIIGGLGNQMFQYAAAKSLAVLNNTRVSANVSVFSNYKTHPLRLNKLNCDCEFDFTRDFRLVLSGFPLLGSAFSKKSMLLNHYVEKDLLFDSSFFDLDDNVLLSGYFQSEKYFSNIRELLIQEFSLDDRLTEAELAINNKIESCNSIAIHIRRGDYITDLSANNIHGICSEEYFEKALNYLDSINVLSDPTTTLFIFSDDILWCKDNLAFKYRTVFVEGSVDRPEVDIHLMSKCKHQVISNSTFSWWGAWLNTNLDKCVIAPLKWFNSLHDSTDIVPKQWMRL

SEQ ID NO: 11 - DNA, 873 bp, Pseudohalocynthiibacter aestuariivivens
  source 1..873: mol_type = genomic DNA
atgaatgagagcgatccgggtcgtatgattaccacccgtctgttcggcggtgcgggcaaccaactgttccaatatgcggcgggtcgtgcgctggcggatcacctgggttgcgaactggcgattgacagccgttacgttgcgggtagccacgaccgtggtgattgctttgcgcacttcggtcaggcgcgttttgcgcgtgagattcgtctgccgccggttaaagcggatggtgttctgcgttacgcgctgtggcgtaagttcggtcgtgcgccgcgtttttaccgtgaacgtggcctgggtttcgatccgagctttttcgatctgccgcgtggtacctatctgcacggttattggcagagcccgcgttatttcgcgccgatcgcgggtcaactgcgtcgtgatctgatgttcaccagcagcctggatgcgaaaaacaccgacatggcggcgcgtattgcgaccgcggcgatgccggttagcctgcacgttcgtcgtggtgattacatcgcgggtgacagctacgcggcgtgcccgccggactattaccgtcgtgcggttagctgcatcgcggaaaacgcggcgcaaccgctgacctgctttgtgttcagcaacgatccggactgggcgcgtgacaacctggatctgggtcaagagaccgttatcgtggatctgaacgacgaaaccaccggtcacttcgatatggcgctgatggcgcgttgcacccacaacatcattgcgaacagcacctttagctggtggggtgcgtggctgaacccgcaaccgaacaagaccgtgattgcgccggcggcgtggtttgcgaaagataaactgcataacccggacctgtgcccgccggagtgggtgcgtctgtaa

SEQ ID NO: 12 - protein, 290 aa, Pseudohalocynthiibacter aestuariivivens
MNESDPGRMITTRLFGGAGNQLFQYAAGRALADHLGCELAIDSRYVAGSHDRGDCFAHFGQARFAREIRLPPVKADGVLRYALWRKFGRAPRFYRERGLGFDPSFFDLPRGTYLHGYWQSPRYFAPIAGQLRRDLMFTSSLDAKNTDMAARIATAAMPVSLHVRRGDYIAGDSYAACPPDYYRRAVSCIAENAAQPLTCFVFSNDPDWARDNLDLGQETVIVDLNDETTGHFDMALMARCTHNIIANSTFSWWGAWLNPQPNKTVIAPAAWFAKDKLHNPDLCPPEWVRL

SEQ ID NO: 13 - DNA, 882 bp, Sterolibacteriaceae bacterium J5B
  source 1..882: mol_type = genomic DNA
atgattattgtgcgtctgtgcggcggtctgggtaaccaaatgtttcagtatgcggcgggtctggcgctgagcctgcgtcacggtgttccgctgcgttttgatctggaatggttcgaccgtgttcacctgcaccaaggtctggaactggatcgtgttttcggtctggatctgccgcgtgcgaccccgagcgaaatgcgtcaagttctgggtggctttagccacccgctggcgcgtcgtctggtggttcgtaagcgtctgcgttggctgctgccggcgagctacgcgctggagccgtatttccactactggccgggtttcgaaaccctgggtccgaacgcgtacctggatggttactggcagagcgaacgttacttccagcgtcacgcgggtagcgttcgtgcggcgttccgttttgcggttgcgctggatgagcgtaaccgtaccctgatggaagagatggcgatgcacgaaagcgttagcgtgcacgttcgtcgtggtgacttcgttcaggatccggtggttcgtcgtgtgcacggtgttgacctgaccgcgtactatccgcaagcgctggcggttatgatgggtcgtctgcgtaacccgcacttctacgtgttcagcgacgatccggaatgggttcgtggtaacctgcgtctgagcgcgccgctgaccatcgttgagcacaaccgtggcaaaaacagctaccgtgacatgcagctgatgagcgcgtgccgtcaccacgttctggcgaacagcagcttcagctggtggggtgcgtggctgaaccaatggcgtgataagatcgttgtggcgccgaagcagtggtttaaggttcgtgactttgacacccgtgatctgtatagcccgggttggattgtgctgtaa

SEQ ID NO: 14 - protein, 293 aa, Sterolibacteriaceae bacterium J5B
MIIVRLCGGLGNQMFQYAAGLALSLRHGVPLRFDLEWFDRVHLHQGLELDRVFGLDLPRATPSEMRQVLGGFSHPLARRLVVRKRLRWLLPASYALEPYFHYWPGFETLGPNAYLDGYWQSERYFQRHAGSVRAAFRFAVALDERNRTLMEEMAMHESVSVHVRRGDFVQDPVVRRVHGVDLTAYYPQALAVMMGRLRNPHFYVFSDDPEWVRGNLRLSAPLTIVEHNRGKNSYRDMQLMSACRHHVLANSSFSWWGAWLNQWRDKIVVAPKQWFKVRDFDTRDLYSPGWIVL

SEQ ID NO: 15 - DNA, 855 bp, Pedobacter sp. CF074
  source 1..855: mol_type = genomic DNA
atgaaaattatcaaaatcctgggtggtctgggaaatcaaatgtttcagtatgcgttctacttgtccatggcaaatcgcttcaaacatgtgaaagcggatattaaccactttgaaaactatgacttgcataatggcttcgaaatcgagaaggtctttggcgttaagattaacaaagctagctcctttctggtgaaaatctttgacaaagaaaattctgcgtggaaatatcgcaaattacgccgcattatgggtactaagaacgccgtcttggatgaaaagaaggaatttgtgttcgataacgacattctgaataatgccaagaacctcatgtatcgcggctactggcagaacgagaaatactttctggagattagcgacaaaattcggagtgcctttacctttcagaaacctctggtagcggaaaatctgaaaatttcgaaactgattcagaaaacggaaagtgtcagcttacacattcgtcgtggtgattatgttgggcattccttacttggtggcatttgcgatctcaattactataagaacgcgattagcattatttatgggaaagtagcgaaaccgaccttctttgtgttctctaatgacatcacatggtgtaaacagaacctgaaaattgaagctgccaattacatctcgtggaaccaaggcagtgattcgtacaaagatatgcaacttatgagcctgtgtaaacacaatgtgatcgcaaactcatcattctcttggtggggagcttggctgaacaacaaccagaacaaaatcgttatcgcaccgaaacgttggacgaatgacccgaattatgatgataccgatatttgcccacatagctggatcaaaatc

SEQ ID NO: 16 - protein, 285 aa, Pedobacter sp. CF074
MKIIKILGGLGNQMFQYAFYLSMANRFKHVKADINHFENYDLHNGFEIEKVFGVKINKASSFLVKIFDKENSAWKYRKLRRIMGTKNAVLDEKKEFVFDNDILNNAKNLMYRGYWQNEKYFLEISDKIRSAFTFQKPLVAENLKISKLIQKTESVSLHIRRGDYVGHSLLGGICDLNYYKNAISIIYGKVAKPTFFVFSNDITWCKQNLKIEAANYISWNQGSDSYKDMQLMSLCKHNVIANSSFSWWGAWLNNNQNKIVIAPKRWTNDPNYDDTDICPHSWIKI

SEQ ID NO: 17 - DNA, 864 bp, Neisseriales bacterium
  source 1..864: mol_type = other DNA
atgaataatatcatcgtgaaatgtcttggtggcctgggtaaccagatgtttcaatacgccttttatcgccgcttacagctggaaaataagaacgtctttctggatatttcggggttcaaagactacagtctgcactatggctttgaactgaaccgtgtgttcaaactgaatgtggatgaacccgattgtagcctggttgatgaaatcaagaaatactctatgagtcgtgggttatggtatcgcatttgtcgcaaactgaagctctataaccagtatattacgcagaagaatttcaactacgatccgcaatatgtgagtttcacgaataaccaaaccgtttatctcgatggttattggcaaagcgagaaatacttcggagtacattcggataccatccggaacgattttaaatttccgcagttggatgttcagaacaagaaatatgcggacaaaatccagttggcgaaatccgtgagcattcacattcgtatgggagactatgtggatcatcctattcatggcggcatttgcactattgactactaccaacgtgctattgagttcattcgctctaaactggataacccgacattctttgtctttagcaatgacgttgaatggtgcaaacagaaccttaatatcagcgactgcatttacattgccgataatgtcggcgaaaatagctatcgcgacatgcagttaatgtccttgtgcaaacacaacatcattgcgaattcatcgttttcctggtggggtgcatggctgaactctaactcggataaaatcgtaatcgcaccgtcaaaatggtttaacgacccaaccatcaacaccaaagatctgctgccaaattcatggattcagatc

SEQ ID NO: 18 - protein, 288 aa, Neisseriales bacterium
MNNIIVKCLGGLGNQMFQYAFYRRLQLENKNVFLDISGFKDYSLHYGFELNRVFKLNVDEPDCSLVDEIKKYSMSRGLWYRICRKLKLYNQYITQKNFNYDPQYVSFTNNQTVYLDGYWQSEKYFGVHSDTIRNDFKFPQLDVQNKKYADKIQLAKSVSIHIRMGDYVDHPIHGGICTIDYYQRAIEFIRSKLDNPTFFVFSNDVEWCKQNLNISDCIYIADNVGENSYRDMQLMSLCKHNIIANSSFSWWGAWLNSNSDKIVIAPSKWFNDPTINTKDLLPNSWIQI

SEQ ID NO: 19 - DNA, 876 bp, Candidatus Methylobacter favarea
  source 1..876: mol_type = genomic DNA
atgatcatttcgcagatcattggcggtttaggcaaccagatgttccagtatgctgctgcacgcagcttgtctgtcgaacggaatcaaccgctccgtctgaatattgccgagtttgacggctacgggttacatcagggcttcgaactggaacgcgtgtttaactgtcccgcagaaattgcgaccaaagcagaagtcgggtccattctgggctggcagttctttagcgtgattcgccgcgtactggctcgtccaggtatggcggcgttgcgccgtgatggttttgtggtggaaccacacttccactattggccggaaatcaatcggattccgaaggattgctatctggtaggctattggcaaagtgagcgctacttcgagaaacatgcgagcgaaatccgtgccgattttgcgttcaaacttccgctgagtgatcgtaactcgattctgtcagagcagatttcccaggttaatgcggtttcccttcatgttcgccgtggcgattatgcgaagaacagcaaaactcgtgctcgccatggtttgtgctcaccggactactatcagcgtgccattaattacatctctggacaagtcgaacaaccccgcttctttatcttctcggatgatatggcatgggtgaaaacgcacctgaaaatggcctttccgtgctactatgtcgatcacaatcgcaacgaagagtcttacaatgacatgcatctgatgtcactctgtcgccatcacatcattgccaacagcagctttagttggtggggagcgtggctgaatccggcgccagacaaaatcgtggttgcaccggtaaaatggtttgccgacaagaacaacaacaaagatctgtttcctcctggttgggtgacctta

SEQ ID NO: 20 - protein, 292 aa, Candidatus Methylobacter favarea
MIISQIIGGLGNQMFQYAAARSLSVERNQPLRLNIAEFDGYGLHQGFELERVFNCPAEIATKAEVGSILGWQFFSVIRRVLARPGMAALRRDGFVVEPHFHYWPEINRIPKDCYLVGYWQSERYFEKHASEIRADFAFKLPLSDRNSILSEQISQVNAVSLHVRRGDYAKNSKTRARHGLCSPDYYQRAINYISGQVEQPRFFIFSDDMAWVKTHLKMAFPCYYVDHNRNEESYNDMHLMSLCRHHIIANSSFSWWGAWLNPAPDKIVVAPVKWFADKNNNKDLFPPGWVTL

SEQ ID NO: 21 - DNA, 909 bp, Escherichia coli O86
  source 1..909: mol_type = genomic DNA
atgtatagttgtttgtctggtggattaggtaatcaaatgtttcagtatgctgcggcatatatcttacagagaaagcttaaacaaagatcattagttttagacgatagctattttttagattgctcaaatcgtgatacacgtagaagatttgaattgaatcaatttaacatatgttatgatcgtctgactacaagtaaggaaaaaaaagagatatccataatacgacatgtaaatagatatcgtttgcccttatttgttacaaattctatatttggagttctactaaaaaaaaactatttgcctgaagcaaaattttatgaatttttgaacaactgtaaattacaggttaaaaatggttattgtctattttcttatttccaggatgctacattgatagatagtcatcgtgatatgattctcccattattccagattaatgaagatttgctccacttatgtaatgacttgcatatttacaaaaaagtgatatgtgagaatgctaacacaacttcactacatatcaggcgtggagactacatcaccaaccctcacgcctctaaatttcatggggtgttgcccatggattactatgaaaaggctattcgttatattgaggatgttcaaggagaacaggtgattatcgtattttcagatgatgtgaaatgggctgagaatacatttgctaatcaacctaattattacgttgttaataattctgaatgcgagtacagtgcgattgatatgtttttaatgtcaaagtgtaaaaacaatataatagccaatagtacatatagttggtggggggcatggttaaatactttcgaagataaaatagttgtttcccctcgtaagtggtttgctggaaataataaatctaagttgaccatggatagttggattaatctttga

SEQ ID NO: 22 - protein, 302 aa, Escherichia coli O86
MYSCLSGGLGNQMFQYAAAYILQRKLKQRSLVLDDSYFLDCSNRDTRRRFELNQFNICYDRLTTSKEKKEISIIRHVNRYRLPLFVTNSIFGVLLKKNYLPEAKFYEFLNNCKLQVKNGYCLFSYFQDATLIDSHRDMILPLFQINEDLLHLCNDLHIYKKVICENANTTSLHIRRGDYITNPHASKFHGVLPMDYYEKAIRYIEDVQGEQVIIVFSDDVKWAENTFANQPNYYVVNNSECEYSAIDMFLMSKCKNNIIANSTYSWWGAWLNTFEDKIVVSPRKWFAGNNKSKLTMDSWINL

SEQ ID NO: 23 - DNA, 897 bp, Escherichia coli O127
  source 1..897: mol_type = genomic DNA
atgtattgctgtctatccggtgggttaggtaatcaaatgttccaatatgctgcagcctatatccttaagcaacattttcctgatactatattagtgcttgatgatagttattatttcaaccagcctcaaaaagatactatacgacatcttgagcttgatcaatttaaaattatttttgataggtttagttctaaagatgaaaaagtaaaaataaatcgtttgaggaaacataaaaaaataccactgcttaacagttttcttcagttcactgcaattaaactgtgtaataaatattcattaaatgatgcttcttattacaatccggaatcaattaaaaacattgatgttgcgtgtctattctcattttaccaagattctaaattattaaatgaacatagggatttaattttgcccctttttgaaatacgtgatgatcttcgcgtgttatgtcataacctacaaatatattccttaattactgactctaagaatataacgtcaattcatgtgcgacgtggagattatgtaaataataaacatgctgcaaaatttcacggcactctaagtatggattattatattagtgcaatggaatacattgaaagtgaatgtggctctcagacatttataatctttacagatgatgtcatatgggcaaaggaaaaattctcaaaatatagcaattgcttggttgctgatgctgatgaaaacaaatttagtgtaattgatatgtatttaatgtcattgtgtaataataatattattgcaaacagcacatatagttggtggggggcatggctaaacaggtcagaagataagctagtcatcgcgcctaaacaatggtacatatccggaaatgaatgctctcttaaaaatgaaaactggatagcaatgtag

SEQ ID NO: 24 - protein, 298 aa, Escherichia coli O127
MYCCLSGGLGNQMFQYAAAYILKQHFPDTILVLDDSYYFNQPQKDTIRHLELDQFKIIFDRFSSKDEKVKINRLRKHKKIPLLNSFLQFTAIKLCNKYSLNDASYYNPESIKNIDVACLFSFYQDSKLLNEHRDLILPLFEIRDDLRVLCHNLQIYSLITDSKNITSIHVRRGDYVNNKHAAKFHGTLSMDYYISAMEYIESECGSQTFIIFTDDVIWAKEKFSKYSNCLVADADENKFSVIDMYLMSLCNNNIIANSTYSWWGAWLNRSEDKLVIAPKQWYISGNECSLKNENWIAM

SEQ ID NO: 25 - DNA, 861 bp, Helicobacter mustelae ATCC43772
  source 1..861: mol_type = genomic DNA
atggattttaagattgtgcaagtgcatggaggacttggaaatcagatgtttcaatacgcttttgccaagagtttgcaaacacatctcaatatacccgtgctacttgataccacctggtttgattatggcaatcgggaattgggattgcatctttttcccatcgatttgcaatgtgctagtgcacagcaaattgctgctgcccatatgcaaaacctgccaaggctagtgagaggtgcgctcagacgtatgggtctaggcagagtcagcaaggaaatcgtgtttgaatacatgccagagctgtttgagccaagtcgcattgcttattttcatggctatttccaagatccaagatattttgaagacatctctcccctgattaagcaaacattcaccctgcctcaccccacagagcatgcagagcaatatagccgcaaactctctcagattttggcggcaaaaaatagcgtatttgtgcatataaggcgaggggattatatgagacttggctggcaacttgatatcagctaccaactacgcgccattgcatatatggccaagcgcgtgcaaaatttggagctatttttattttgcgaggatttggaatttgtgcagaatcttgatcttggctatccctttgtggatatgaccacaagggatggggcggcgcattgggatatgatgctgatgcaatcttgcaagcatggcattatcacaaatagtacctatagttggtgggcggcatatttgataaaaaatccagaaaaaatcattattggaccaagccactggatctatggcaatgaaaatatcctttgcaaggattgggtgaagatagaatcccaatttgagacaaaatcttga

SEQ ID NO: 26 - protein, 286 aa, Helicobacter mustelae ATCC43772
MDFKIVQVHGGLGNQMFQYAFAKSLQTHLNIPVLLDTTWFDYGNRELGLHLFPIDLQCASAQQIAAAHMQNLPRLVRGALRRMGLGRVSKEIVFEYMPELFEPSRIAYFHGYFQDPRYFEDISPLIKQTFTLPHPTEHAEQYSRKLSQILAAKNSVFVHIRRGDYMRLGWQLDISYQLRAIAYMAKRVQNLELFLFCEDLEFVQNLDLGYPFVDMTTRDGAAHWDMMLMQSCKHGIITNSTYSWWAAYLIKNPEKIIIGPSHWIYGNENILCKDWVKIESQFETKS

SEQ ID NO: 27 - DNA, 879 bp, Sideroxydans lithotrophicus ES-11
  source 1..879: mol_type = genomic DNA
atggttattagcaatatcatcggtggtctgggcaatcaaatgtttcagtatgcggcggcgcgtgcgctgagcctgaagctggaagttccgctgaaactggacatcagcggtttcaccaactacgcgctgcaccaaggtttcgaactggatcgtatcttcggttgcaagatcgagattgcgagcgaagcggatgttcacgagattctgggttggcagagcgcgagcggtatccgtcgtgttgtgagccgtccgggtatgagcatcttccgtcgtaagggtttcgtggttgaaccgcacttcagctactggaacggtattcgtaaaatcaccggtgattgctacctggcgggttattggcagagcgagaaatacttcctggatgcggcggttgaaatccgtaaggactttagcttcaagctgccgctggacagccacaacgcggagctggcggaaaagatcgatcaggagaacgcggttagcctgcacattcgtcgtggtgattacgcgaacaacccgctgaccgcggcgacccacggtctgtgcagcctggactactatcgtaaaagcattaagcacatcgcgggtcaagttcgtaacccgtacttctttgtgttcagcgatgacatcgcgtgggttaaagacaacctggagatcgaattcccgagccagtatgtggactacaaccacggtagcatgagcttcaacgacatgcgtctgatgagcctgtgcaaacaccacatcattgcgaacagcagcttcagctggtggggtgcgtggctgaacccgaacccggaaaaggtggttatcgcgccggagcgttggtttgcgaatcgtaccgacgttcaagacctgctgccgccgggttgggttaagctgtaa

SEQ ID NO: 28 - protein, 292 aa, Sideroxydans lithotrophicus ES-11
MVISNIIGGLGNQMFQYAAARALSLKLEVPLKLDISGFTNYALHQGFELDRIFGCKIEIASEADVHEILGWQSASGIRRVVSRPGMSIFRRKGFVVEPHFSYWNGIRKITGDCYLAGYWQSEKYFLDAAVEIRKDFSFKLPLDSHNAELAEKIDQENAVSLHIRRGDYANNPLTAATHGLCSLDYYRKSIKHIAGQVRNPYFFVFSDDIAWVKDNLEIEFPSQYVDYNHGSMSFNDMRLMSLCKHHIIANSSFSWWGAWLNPNPEKVVIAPERWFANRTDVQDLLPPGWVKL

SEQ ID NO: 29 - DNA, 882 bp, Thermosynechococcus elongatus BP-1
  source 1..882: mol_type = genomic DNA
atgattatcgttcacctgtgcggcggcctgggcaaccaaatgtttcaatacgcggcgggtctggcggcggcgcatcgcatcggcagcgaggtgaagttcgatacccactggtttgacgcgacctgcctgcaccaaggtctggagctgcgtcgtgtgtttggtctggaactgccggaaccgagcagcaaggatctgcgtaaggttctgggtgcgtgcgttcacccggcggttcgtcgtctgctggcgggtcactttctgcacggtctgcgtccgaaaagcctggtgatccaaccgcactttcactactggaccggttttgagcacctgccggataacgtgtacctggaaggttactggcaaagcgaacgttacttcagcaacatcgcggacattatccgtcagcaattccgttttgtggaaccgctggacccgcacaacgcggcgctgatggacgagatgcaaagcggtgtgagcgttagcctgcacattcgtcgtggtgactacttcaacaacccgcaaatgcgtcgtgttcacggtgttgatctgagcgaatactatccggcggcggttgcgaccatgatcgagaagaccaacgcggaacgtttttacgtgttcagcgatgacccgcaatgggttctggaacacctgaaactgccggttagctataccgtggttgatcacaaccgtggtgcggcgagctatcgtgacatgcaactgatgagcgcgtgccgtcaccacatcattgcgaacagcacctttagctggtggggtgcgtggctgaacccgcgtccggataaggtggttattgcgccgcgtcactggtttaatgttgatgtttttgacacccgtgacctgtattgcccgggttggattgttctgtaa

SEQ ID NO: 30 - protein, 293 aa, Thermosynechococcus elongatus BP-1
MIIVHLCGGLGNQMFQYAAGLAAAHRIGSEVKFDTHWFDATCLHQGLELRRVFGLELPEPSSKDLRKVLGACVHPAVRRLLAGHFLHGLRPKSLVIQPHFHYWTGFEHLPDNVYLEGYWQSERYFSNIADIIRQQFRFVEPLDPHNAALMDEMQSGVSVSLHIRRGDYFNNPQMRRVHGVDLSEYYPAAVATMIEKTNAERFYVFSDDPQWVLEHLKLPVSYTVVDHNRGAASYRDMQLMSACRHHIIANSTFSWWGAWLNPRPDKVVIAPRHWFNVDVFDTRDLYCPGWIVL

SEQ ID NO: 31 - DNA, 903 bp, Helicobacter pylori 26695
  source 1..903: mol_type = genomic DNA
atggcttttaaggtggtgcaaatttgcggagggcttgggaatcaaatgtttcaatacgctttcgctaaaagtttgcaaaaacactctaatacgcctgtgctgttagatatcacttcttttgattggagcgataggaaaatgcaattagaacttttccctattgatttgccctatgcgagcgcgaaagaaatcgctatagctaaaatgcaacacctccccaagctagtaagagacgcgctcaaatgcatgggatttgatagggtgagtcaagaaatcgtttttgaatacgagcctaaattgctaaagccaagccgcttgacttatttttttggctatttccaagatccacgatactttgatgctatatcccctttaatcaagcaaaccttcactctaccaccaccaccagaaaataataagaataataataaaaaagaggaagaatatcagtgcaagctttctttgattttagccgctaaaaacagcgtgtttgtgcatataagaagaggggattatgtggggattggctgtcagcttggtattgactatcaaaaaaaggcgcttgagtatatggcaaagcgcgtgccaaacatggagctttttgtgttttgcgaagacttagaattcacgcaaaatcttgatcttggctacccttttatggacatgaccactagggataaagaagaagaggcgtattgggacatgctgctcatgcaatcttgtcagcatggcattatcgctaatagcacttatagctggtgggcggcctatttgatagaaaatccagaaaaaatcattattggccccaaacactggctttttgggcatgagaatatcctttgtaaggagtgggtgaaaatagaatcccattttgaggtaaaatcccaaaagtataacgcttaa

SEQ ID NO: 32 - protein, 300 aa, Helicobacter pylori 26695
MAFKVVQICGGLGNQMFQYAFAKSLQKHSNTPVLLDITSFDWSDRKMQLELFPIDLPYASAKEIAIAKMQHLPKLVRDALKCMGFDRVSQEIVFEYEPKLLKPSRLTYFFGYFQDPRYFDAISPLIKQTFTLPPPPENNKNNNKKEEEYQCKLSLILAAKNSVFVHIRRGDYVGIGCQLGIDYQKKALEYMAKRVPNMELFVFCEDLEFTQNLDLGYPFMDMTTRDKEEEAYWDMLLMQSCQHGIIANSTYSWWAAYLIENPEKIIIGPKHWLFGHENILCKEWVKIESHFEVKSQKYNA

SEQ ID NO: 33 - DNA, 789 bp, Chromobacterium violaceum ATCC553
  source 1..789: mol_type = genomic DNA
atggacaccatcatgattaaacgtccgctggttagcgttattctgccggtgaataaaaacaatccgcatctggaagaagcaatccagagcattaaaaaccagacctataaagagctggaactgatcattattgccaacaactgcgaggataacttttatagcctgctgctgaaatatcaggaccagaaaaccaaaattatccgcaccagcatcaaatatctgccgtttagcctgaatctgggtgttcatctgagccagggtgaatatattgcacgtatggattcagatgatatcagcgttctggatcgcattgaaaaacaggttaaacgctttctgaatacaccggaactgagcattctgggtagcaatgttgaatatatcaatgaagccagcgaaagcattggctatagcaactatccgctggatcatagcagcattgttaatagctttccgtttcgttgtaatctggcacatccgaccattatggttaaaaaagaagtgattaccacgcttggtggctatatgtatggtagcctgagcgaagattatgatctgtggattcgtgcaagccgtcatggcaatttcaaatttagcaatattgatgaaccgctgctgaagtaccgtattcataaaggtcaggcaaccaataaaagcaacgcctataacatctttgcctttgatagcagcctgaaaatccgtgaatttctgctgaatggtaatgtgcagtatctgctgggtgcagcacgtggtttttttgcatttctgtatgtgcgcttcatcaaaaaatga

SEQ ID NO: 34 - protein, 262 aa, Chromobacterium violaceum ATCC553
MDTIMIKRPLVSVILPVNKNNPHLEEAIQSIKNQTYKELELIIIANNCEDNFYSLLLKYQDQKTKIIRTSIKYLPFSLNLGVHLSQGEYIARMDSDDISVLDRIEKQVKRFLNTPELSILGSNVEYINEASESIGYSNYPLDHSSIVNSFPFRCNLAHPTIMVKKEVITTLGGYMYGSLSEDYDLWIRASRHGNFKFSNIDEPLLKYRIHKGQATNKSNAYNIFAFDSSLKIREFLLNGNVQYLLGAARGFFAFLYVRFIKK

SEQ ID NO: 35 - DNA, 1041 bp, Neisseria polysaccharea ATCC43768
  source 1..1041: mol_type = genomic DNA
atgcagccgctggtgagcgttctgatttgcgcgtacaacgtggagaagtattttgcgcaggcgctggatgcggtggttggtcaaacctggcgtaacctggacatcctgattgttgacgatggcagcaccgatggtaccctggcgatcgcgaaggactttcaaaaacgtgatagccgtatcaagattctggcgcaggcgcaaaacagcggcctgatcccgagcctgaacattggtctggatgagctggcgaaaagcggtggcggtgaatacattgcgcgtaccgatgcggatgatattgcggcgccggattggatcgagaagattgtgggcgagatggaaaaagaccgtagcatcattgcgatgggtgcgtggctggaagttctgagcgaggaaaaggatggcaaccgtctggcgcgtcaccacgagcacggtaaaatttggaagaaaccgacccgtcacgaagacatcgcggcgttctttccgttcggcaacccgatccacaacaacaccatgattatgcgtcgtagcgtgatcgacggcggtctgcgttacaacaccgagcgtgactgggcggaagattaccagttttggtatgatgttagcaagctgggtcgtctggcgtactatccggaggcgctggtgaagtatcgtctgcacgcgaaccaagttagcagcaaacacagcattcgtcaacacgaaatcgcgcagggcattcaaaagaccgcgcgtaacgacttcctgcagagcatgggtttcaaaacccgttttgatagcctggagtaccgtcaaaccaaggcggcggcgtatgagctgctggaaaaagacctgccggaggaagatttcgaacgtgcgcgtcgtttcctgtaccagtgctttaaacgtaccgacaccccgccggcgggtgcgtggctggactttgcggcggatggtcgtatgcgtcgtctgttcaccctgcgtcaatattttagcatcctgcaccgtctgattaagaaccgtcgtcaggcgcgtagcgatagcgcgggtaaagagcaagaaatctaa

SEQ ID NO: 36 - protein, 346 aa, Neisseria polysaccharea ATCC43768
MQPLVSVLICAYNVEKYFAQALDAVVGQTWRNLDILIVDDGSTDGTLAIAKDFQKRDSRIKILAQAQNSGLIPSLNIGLDELAKSGGGEYIARTDADDIAAPDWIEKIVGEMEKDRSIIAMGAWLEVLSEEKDGNRLARHHEHGKIWKKPTRHEDIAAFFPFGNPIHNNTMIMRRSVIDGGLRYNTERDWAEDYQFWYDVSKLGRLAYYPEALVKYRLHANQVSSKHSIRQHEIAQGIQKTARNDFLQSMGFKTRFDSLEYRQTKAAAYELLEKDLPEEDFERARRFLYQCFKRTDTPPAGAWLDFAADGRMRRLFTLRQYFSILHRLIKNRRQARSDSAGKEQEI

SEQ ID NO: 37 - DNA, 20 bp, synthetic construct
  misc_feature 1..20: note = Description of the artificial sequence: base sequence foramplification of catsacB fragment
  source 1..20: mol_type = other DNA
accaggcgtttaagggcacc

SEQ ID NO: 38 - DNA, 21 bp, synthetic construct
  misc_feature 1..21: note = Description of the artificial sequence: base sequence foramplification of catsacB fragment
  source 1..21: mol_type = other DNA
tacggttagccatttgcctgc

SEQ ID NO: 39 - DNA, 42 bp, synthetic construct
  misc_feature 1..42: note = Description of the artificial sequence: base sequence foramplification of lacZ upstream 1
  source 1..42: mol_type = other DNA
ggtgcccttaaacgcctggtagctgtttcctgtgtgaaattg

SEQ ID NO: 40 - DNA, 18 bp, synthetic construct
  misc_feature 1..18: note = Description of the artificial sequence: base sequence foramplification of lacZ upstream 1
  source 1..18: mol_type = other DNA
ccagtctggccctgcacg

SEQ ID NO: 41 - DNA, 43 bp, synthetic construct
  misc_feature 1..43: note = Description of the artificial sequence: base sequence foramplification of lacY downstream1
  source 1..43: mol_type = other DNA
gcaggcaaatggctaaccgtacgaccaacatatcataacggag

SEQ ID NO: 42 - DNA, 20 bp, synthetic construct
  misc_feature 1..20: note = Description of the artificial sequence: base sequence foramplification of lacY downstream1
  source 1..20: mol_type = other DNA
gtttccgctctgtttgctgc

SEQ ID NO: 43 - DNA, 42 bp, synthetic construct
  misc_feature 1..42: note = Description of the artificial sequence: base sequence foramplification oflacZ upstream 2
  source 1..42: mol_type = other DNA
ccgttatgatatgttggtcgagctgtttcctgtgtgaaattg

SEQ ID NO: 44 - DNA, 22 bp, synthetic construct
  misc_feature 1..22: note = Description of the artificial sequence: base sequence foramplification oflacY downstream2
  source 1..22: mol_type = other DNA
cgaccaacatatcataacggag

SEQ ID NO: 45 - DNA, 41 bp, synthetic construct
  misc_feature 1..41: note = Description of the artificial sequence: base sequence foramplification of wcaJ upstream1
  source 1..41: mol_type = other DNA
ggtgcccttaaacgcctggtcgttgttcctgttattagccc

SEQ ID NO: 46 - DNA, 20 bp, synthetic construct
  misc_feature 1..20: note = Description of the artificial sequence: base sequence foramplification of wcaJ upstream1
  source 1..20: mol_type = other DNA
acgcggtcgctatcagcaaa

SEQ ID NO: 47 - DNA, 44 bp, synthetic construct
  misc_feature 1..44: note = Description of the artificial sequence: base sequence foramplification of wcaM downstream1
  source 1..44: mol_type = other DNA
gcaggcaaatggctaaccgtaatttgcgaccattcctggaaaaa

SEQ ID NO: 48 - DNA, 23 bp, synthetic construct
  misc_feature 1..23: note = Description of the artificial sequence: base sequence foramplification of wcaM downstream1
  source 1..23: mol_type = other DNA
acttcacaaacgcctgcatatag

SEQ ID NO: 49 - DNA, 41 bp, synthetic construct
  misc_feature 1..41: note = Description of the artificial sequence: base sequence foramplification of wcaJ upstream2
  source 1..41: mol_type = other DNA
ttccaggaatggtcgcaaatcgttgttcctgttattagccc

SEQ ID NO: 50 - DNA, 23 bp, synthetic construct
  misc_feature 1..23: note = Description of the artificial sequence: base sequence foramplification of wcaM downstream2
  source 1..23: mol_type = other DNA
atttgcgaccattcctggaaaaa

SEQ ID NO: 51 - DNA, 38 bp, synthetic construct
  misc_feature 1..38: note = Description of the artificial sequence: base sequence foramplification of Cvbeta3galT fragment
  source 1..38: mol_type = other DNA
gaggagaaattaaccatggacaccatcatgattaaacg

SEQ ID NO: 52 - DNA, 60 bp, synthetic construct
  misc_feature 1..60: note = Description of the artificial sequence: base sequence foramplification of Cvbeta3galT fragment
  source 1..60: mol_type = other DNA
caccagcggctgcatggttaatttctcctctttaattcattttttgatgaagcgcacata

SEQ ID NO: 53 - DNA, 19 bp, synthetic construct
  misc_feature 1..19: note = Description of the artificial sequence: base sequence foramplification of NplgtAfragment
  source 1..19: mol_type = other DNA
atgcagccgctggtgagcg

SEQ ID NO: 54 - DNA, 43 bp, synthetic construct
  misc_feature 1..43: note = Description of the artificial sequence: base sequence foramplification of NplgtAfragment
  source 1..43: mol_type = other DNA
aatggatttccttacgcgaattagatttcttgctctttacccg

SEQ ID NO: 55 - DNA, 23 bp, synthetic construct
  misc_feature 1..23: note = Description of the artificial sequence: base sequence foramplification of lacY fragment
  source 1..23: mol_type = other DNA
ttcgcgtaaggaaatccattatg

SEQ ID NO: 56 - DNA, 38 bp, synthetic construct
  misc_feature 1..38: note = Description of the artificial sequence: base sequence foramplification of lacY fragment
  source 1..38: mol_type = other DNA
atggtgatggtgatgttaagcgacttcattcacctgac

SEQ ID NO: 57 - DNA, 24 bp, synthetic construct
  misc_feature 1..24: note = Description of the artificial sequence: base sequence foramplification of pUAKQE fragment
  source 1..24: mol_type = other DNA
ggttaatttctcctctttaatatc

SEQ ID NO: 58 - DNA, 22 bp, synthetic construct
  misc_feature 1..22: note = Description of the artificial sequence: base sequence foramplification of pUAKQE fragment
  source 1..22: mol_type = other DNA
catcaccatcaccatcactaag

SEQ ID NO: 59 - DNA, 36 bp, synthetic construct
  misc_feature 1..36: note = Description of the artificial sequence: base sequence foramplification of rcsA fragment
  source 1..36: mol_type = other DNA
acacaggaaacagctgcattgagtgagggtatgcca

SEQ ID NO: 60 - DNA, 38 bp, synthetic construct
  misc_feature 1..38: note = Description of the artificial sequence: base sequence foramplification of rcsA fragment
  source 1..38: mol_type = other DNA
acggccagtgaattcttagcgcatgttgacaaaaatac

SEQ ID NO: 61 - DNA, 22 bp, synthetic construct
  misc_feature 1..22: note = Description of the artificial sequence: base sequence foramplification of pSTV29 fragment
  source 1..22: mol_type = other DNA
agctgtttcctgtgtgaaattg

SEQ ID NO: 62 - DNA, 20 bp, synthetic construct
  misc_feature 1..20: note = Description of the artificial sequence: base sequence foramplification of pSTV29 fragment
  source 1..20: mol_type = other DNA
gaattcactggccgtcgttt

SEQ ID NO: 63 - DNA, 34 bp, synthetic construct
  misc_feature 1..34: note = Description of the artificial sequence: base sequence foramplification of GsFucT fragment
  source 1..34: mol_type = other DNA
acacaggaaacagctatgagcaagaagaagccgg

SEQ ID NO: 64 - DNA, 39 bp, synthetic construct
  misc_feature 1..39: note = Description of the artificial sequence: base sequence foramplification of GsFucT fragment
  source 1..39: mol_type = other DNA
ggcataccctcactcaatgcttagatacgcacccagtcc

SEQ ID NO: 65 - DNA, 37 bp, synthetic construct
  misc_feature 1..37: note = Description of the artificial sequence: base sequence foramplification of FsFucT fragment
  source 1..37: mol_type = other DNA
acacaggaaacagctatgaaagttgtgaaaatccaag

SEQ ID NO: 66 - DNA, 37 bp, synthetic construct
  misc_feature 1..37: note = Description of the artificial sequence: base sequence foramplification of FsFucT fragment
  source 1..37: mol_type = other DNA
ggcataccctcactcaatgcttagattttgatccagc

SEQ ID NO: 67 - DNA, 36 bp, synthetic construct
  misc_feature 1..36: note = Description of the artificial sequence: base sequence foramplification of NbFucT1 fragment
  source 1..36: mol_type = other DNA
acacaggaaacagctatgcaaatcgtgtggtgcctg

SEQ ID NO: 68 - DNA, 40 bp, synthetic construct
  misc_feature 1..40: note = Description of the artificial sequence: base sequence foramplification of NbFucT1 fragment
  source 1..40: mol_type = other DNA
ggcataccctcactcaatgcttagattttcacccagctcg

SEQ ID NO: 69 - DNA, 36 bp, synthetic construct
  misc_feature 1..36: note = Description of the artificial sequence: base sequence foramplification of MtFucT fragment
  source 1..36: mol_type = other DNA
acacaggaaacagctatggttattacccatctgatc

SEQ ID NO: 70 - DNA, 38 bp, synthetic construct
  misc_feature 1..38: note = Description of the artificial sequence: base sequence foramplification of MtFucT fragment
  source 1..38: mol_type = other DNA
ggcataccctcactcaatgcttattgtttaatccagcc

SEQ ID NO: 71 - DNA, 37 bp, synthetic construct
  misc_feature 1..37: note = Description of the artificial sequence: base sequence foramplification of AjFucT fragment
  source 1..37: mol_type = other DNA
acacaggaaacagctatggtgaaaatcaaaatcatcg

SEQ ID NO: 72 - DNA, 39 bp, synthetic construct
  misc_feature 1..39: note = Description of the artificial sequence: base sequence foramplification of AjFucT fragment
  source 1..39: mol_type = other DNA
ggcataccctcactcaatgcttacagacgcatccactgc

SEQ ID NO: 73 - DNA, 35 bp, synthetic construct
  misc_feature 1..35: note = Description of the artificial sequence: base sequence foramplification of PaFucT fragment
  source 1..35: mol_type = other DNA
acacaggaaacagctatgaatgagagcgatccggg

SEQ ID NO: 74 - DNA, 39 bp, synthetic construct
  misc_feature 1..39: note = Description of the artificial sequence: base sequence foramplification of PaFucT fragment
  source 1..39: mol_type = other DNA
ggcataccctcactcaatgcttacagacgcacccactcc

SEQ ID NO: 75 - DNA, 35 bp, synthetic construct
  misc_feature 1..35: note = Description of the artificial sequence: base sequence foramplification of SbFucT fragment
  source 1..35: mol_type = other DNA
acacaggaaacagctatgattattgtgcgtctgtg

SEQ ID NO: 76 - DNA, 38 bp, synthetic construct
  misc_feature 1..38: note = Description of the artificial sequence: base sequence foramplification of SbFucT fragment
  source 1..38: mol_type = other DNA
ggcataccctcactcaatgcttacagcacaatccaacc

SEQ ID NO: 77 - DNA, 34 bp, synthetic construct
  misc_feature 1..34: note = Description of the artificial sequence: base sequence foramplification of PsFucT fragment
  source 1..34: mol_type = other DNA
acacaggaaacagctatgaaaattatcaaaatcc

SEQ ID NO: 78 - DNA, 36 bp, synthetic construct
  misc_feature 1..36: note = Description of the artificial sequence: base sequence foramplification of PsFucT fragment
  source 1..36: mol_type = other DNA
ggcataccctcacgattttgatccagctatgtgggc

SEQ ID NO: 79 - DNA, 37 bp, synthetic construct
  misc_feature 1..37: note = Description of the artificial sequence: base sequence foramplification of NbFucT2 fragment
  source 1..37: mol_type = other DNA
acacaggaaacagctatgaataatatcatcgtgaaat

SEQ ID NO: 80 - DNA, 38 bp, synthetic construct
  misc_feature 1..38: note = Description of the artificial sequence: base sequence foramplification of NbFucT2 fragment
  source 1..38: mol_type = other DNA
ggcataccctcacgatctgaatccatgaatttggcagc

SEQ ID NO: 81 - DNA, 33 bp, synthetic construct
  misc_feature 1..33: note = Description of the artificial sequence: base sequence foramplification of CMfFucT fragment
  source 1..33: mol_type = other DNA
acacaggaaacagctatgatcatttcgcagatc

SEQ ID NO: 82 - DNA, 34 bp, synthetic construct
  misc_feature 1..34: note = Description of the artificial sequence: base sequence foramplification of CMfFucT fragment
  source 1..34: mol_type = other DNA
ggcataccctcactaaggtcacccaaccaggagg

SEQ ID NO: 83 - DNA, 37 bp, synthetic construct
  misc_feature 1..37: note = Description of the artificial sequence: base sequence foramplification of WbwK fragment
  source 1..37: mol_type = other DNA
acacaggaaacagctatgtatagttgtttgtctggtg

SEQ ID NO: 84 - DNA, 38 bp, synthetic construct
  misc_feature 1..38: note = Description of the artificial sequence: base sequence foramplification of WbwK fragment
  source 1..38: mol_type = other DNA
ggcataccctcactcaaagattaatccaactatccatg

SEQ ID NO: 85 - DNA, 37 bp, synthetic construct
  misc_feature 1..37: note = Description of the artificial sequence: base sequence foramplification of WbiQ fragment
  source 1..37: mol_type = other DNA
acacaggaaacagctatgtattgctgtctatccggtg

SEQ ID NO: 86 - DNA, 34 bp, synthetic construct
  misc_feature 1..34: note = Description of the artificial sequence: base sequence foramplification of WbiQ fragment
  source 1..34: mol_type = other DNA
ggcataccctcacctacattgctatccagttttc

SEQ ID NO: 87 - DNA, 35 bp, synthetic construct
  misc_feature 1..35: note = Description of the artificial sequence: base sequence foramplification of HMFT fragment
  source 1..35: mol_type = other DNA
acacaggaaacagctatggattttaagattgtgca

SEQ ID NO: 88 - DNA, 41 bp, synthetic construct
  misc_feature 1..41: note = Description of the artificial sequence: base sequence foramplification of HMFT fragment
  source 1..41: mol_type = other DNA
ggcataccctcactcaatgctcaagattttgtctcaaattg

SEQ ID NO: 89 - DNA, 37 bp, synthetic construct
  misc_feature 1..37: note = Description of the artificial sequence: base sequence foramplification of FucT54 fragment
  source 1..37: mol_type = other DNA
acacaggaaacagctatggttattagcaatatcatcg

SEQ ID NO: 90 - DNA, 39 bp, synthetic construct
  misc_feature 1..39: note = Description of the artificial sequence: base sequence foramplification of FucT54 fragment
  source 1..39: mol_type = other DNA
ggcataccctcactcaatgcttacagcttaacccaaccc

SEQ ID NO: 91 - DNA, 37 bp, synthetic construct
  misc_feature 1..37: note = Description of the artificial sequence: base sequence foramplification of Te2FT fragment
  source 1..37: mol_type = other DNA
acacaggaaacagctatgattatcgttcacctgtgcg

SEQ ID NO: 92 - DNA, 38 bp, synthetic construct
  misc_feature 1..38: note = Description of the artificial sequence: base sequence foramplification of Te2FT fragment
  source 1..38: mol_type = other DNA
ggcataccctcactcaatgcttacagaacaatccaacc

SEQ ID NO: 93 - DNA, 35 bp, synthetic construct
  misc_feature 1..35: note = Description of the artificial sequence: base sequence foramplification of FutC fragment
  source 1..35: mol_type = other DNA
acacaggaaacagctatggcttttaaggtggtgca

SEQ ID NO: 94 - DNA, 38 bp, synthetic construct
  misc_feature 1..38: note = Description of the artificial sequence: base sequence foramplification of FutC fragment
  source 1..38: mol_type = other DNA
ggcataccctcactcaatgcttaagcgttatacttttg

SEQ ID NO: 95 - DNA, 14 bp, synthetic construct
  misc_feature 1..14: note = Description of the artificial sequence: base sequence foramplification of pSTV-rcsA fragment
  source 1..14: mol_type = other DNA
gtgagggtatgcca